European Patent Application EP 4 403 577 A1, published July 24, 2024. Title: Modified Anti-VEGFR2(KDR) Antibody and Use Thereof. Applicant: Pharmabcine Inc. The sequence listing filed with the application follows.

SEQUENCE LISTING (50 sequences)

SEQ ID NO: 1 - protein, 8 aa, synthetic construct
  REGION 1..8: note = Heavy-chain CDR1
GYTFSSYW

SEQ ID NO: 2 - protein, 8 aa, synthetic construct
  REGION 1..8: note = Heavy-chain CDR2
INPGNGHT

SEQ ID NO: 3 - protein, 14 aa, synthetic construct
  REGION 1..14: note = Heavy-chain CDR3
ARHWGPSLTSPFDY

SEQ ID NO: 4 - protein, 6 aa, synthetic construct
  REGION 1..6: note = Light-chain CDR1
NLGDVN

SEQ ID NO: 5 - skipped

SEQ ID NO: 6 - protein, 10 aa, synthetic construct
  REGION 1..10: note = Light-chain CDR3
QAPTRIAPYT

SEQ ID NO: 7 - protein, 8 aa, synthetic construct
  REGION 1..8: note = Heavy-chain CDR1
GYTFSSYW

SEQ ID NO: 8 - protein, 8 aa, synthetic construct
  REGION 1..8: note = Heavy-chain CDR2
INPGNGHT

SEQ ID NO: 9 - protein, 14 aa, synthetic construct
  REGION 1..14: note = Heavy-chain CDR3
ARSYRPSLTSPFDF

SEQ ID NO: 10 - protein, 6 aa, synthetic construct
  REGION 1..6: note = Light-chain CDR1
NLGDVN

SEQ ID NO: 11 - skipped

SEQ ID NO: 12 - protein, 10 aa, synthetic construct
  REGION 1..10: note = Light-chain CDR3
QAPTTNEPYT

SEQ ID NO: 13 - protein, 8 aa, synthetic construct
  REGION 1..8: note = Heavy-chain CDR1
GYTFSSYW

SEQ ID NO: 14 - protein, 8 aa, synthetic construct
  REGION 1..8: note = Heavy-chain CDR2
INPGNGHT

SEQ ID NO: 15 - protein, 14 aa, synthetic construct
  REGION 1..14: note = Heavy-chain CDR3
ARHWGPSLTSPFDY

SEQ ID NO: 16 - protein, 6 aa, synthetic construct
  REGION 1..6: note = Light-chain CDR1
NLGDVN

SEQ ID NO: 17 - skipped

SEQ ID NO: 18 - protein, 10 aa, synthetic construct
  REGION 1..10: note = Light-chain CDR3
QAPTNNDPYT

SEQ ID NO: 19 - protein, 8 aa, synthetic construct
  REGION 1..8: note = Heavy-chain CDR1
GYTFSSYW

SEQ ID NO: 20 - protein, 8 aa, synthetic construct
  REGION 1..8: note = Heavy-chain CDR2
INPGNGHT

SEQ ID NO: 21 - protein, 14 aa, synthetic construct
  REGION 1..14: note = Heavy-chain CDR3
ARHWGPSLTSPFDY

SEQ ID NO: 22 - protein, 6 aa, synthetic construct
  REGION 1..6: note = Light-chain CDR1
NLGDVN

SEQ ID NO: 23 - skipped

SEQ ID NO: 24 - protein, 10 aa, synthetic construct
  REGION 1..10: note = Light-chain CDR3
QAPTTHLPYT

SEQ ID NO: 25 - protein, 8 aa, synthetic construct
  REGION 1..8: note = Heavy-chain CDR1
GYTFSSYW

SEQ ID NO: 26 - protein, 8 aa, synthetic construct
  REGION 1..8: note = Heavy-chain CDR2
INPGNGHT

SEQ ID NO: 27 - protein, 14 aa, synthetic construct
  REGION 1..14: note = Heavy-chain CDR3
ARHWGPSLTSPFDY

SEQ ID NO: 28 - protein, 6 aa, synthetic construct
  REGION 1..6: note = Light-chain CDR1
NLGDVN

SEQ ID NO: 29 - skipped

SEQ ID NO: 30 - protein, 10 aa, synthetic construct
  REGION 1..10: note = Light-chain CDR3
QAPTKNVPYT

SEQ ID NO: 31 - DNA, 363 bp, synthetic construct
  misc_feature 1..363: note = VH
  source 1..363: mol_type = other DNA
gaggtgcagctggtggaatccggcggaggactggtgcagcctggcggctccctgagactgtcttgcgccgcctccggatacaccttcagcagctactggatgagctgggtgcgacaggcccctggcaagggcctcgaatgggtgtcagagattaatcctggcaacggtcatactaactacaacgagaagttcaagtcacggttcaccatctccagagacaagtccaagaacaccctgtacctgcagatgaactccctgcgggccgaggacaccgccgtgtactactgcgccagacattggggcccgagtcttacttctccctttgactactggggccagggcaccctggtgacagtgtcctcc

SEQ ID NO: 32 - protein, 121 aa, synthetic construct
  REGION 1..121: note = VH
EVQLVESGGGLVQPGGSLRLSCAASGYTFSSYWMSWVRQAPGKGLEWVSEINPGNGHTNYNEKFKSRFTISRDKSKNTLYLQMNSLRAEDTAVYYCARHWGPSLTSPFDYWGQGTLVTVSS

SEQ ID NO: 33 - DNA, 330 bp, synthetic construct
  misc_feature 1..330: note = VL
  source 1..330: mol_type = other DNA
gacatccagatgacccagtctccatcctccctgtctgcatctgtaggagacagagtcaccatcacttgccgggcagataaccttggagatgtaaatgtacactggtatcagcagaaaccagggaaagcccctaagctcctgatctattatgatgccgaccggccctcaggggtcccatcaaggttcagtggcagtaattctgggaatgatgccactctcaccatcagcagtctgcaacctgaagattttgcaacttactactgtcaagcgcccacaagaatagcgccttataccttcggccagggcaccaaggtggaaatcaagcggacc

SEQ ID NO: 34 - protein, 110 aa, synthetic construct
  REGION 1..110: note = VL
DIQMTQSPSSLSASVGDRVTITCRADNLGDVNVHWYQQKPGKAPKLLIYYDADRPSGVPSRFSGSNSGNDATLTISSLQPEDFATYYCQAPTRIAPYTFGQGTKVEIKRT

SEQ ID NO: 35 - DNA, 363 bp, synthetic construct
  misc_feature 1..363: note = VH
  source 1..363: mol_type = other DNA
gaggtgcagctggtggaatccggcggaggactggtgcagcctggcggctccctgagactgtcttgcgccgcctccggatacaccttcagcagctactggatgagctgggtgcgacaggcccctggcaagggcctcgaatgggtgtcagagattaatcctggcaacggtcatactaactacaacgagaagttcaagtcacggttcaccatctccagagacaagtccaagaacaccctgtacctgcagatgaactccctgcgggccgaggacaccgccgtgtactactgcgccagaagctaccgcccgagtcttacttctccctttgatttctggggccagggcaccctggtgacagtgtcctcc

SEQ ID NO: 36 - protein, 121 aa, synthetic construct
  REGION 1..121: note = VH
EVQLVESGGGLVQPGGSLRLSCAASGYTFSSYWMSWVRQAPGKGLEWVSEINPGNGHTNYNEKFKSRFTISRDKSKNTLYLQMNSLRAEDTAVYYCARSYRPSLTSPFDFWGQGTLVTVSS

SEQ ID NO: 37 - DNA, 330 bp, synthetic construct
  misc_feature 1..330: note = VL
  source 1..330: mol_type = other DNA
gacatccagatgacccagtctccatcctccctgtctgcatctgtaggagacagagtcaccatcacttgccgggcagataaccttggagatgtaaatgtacactggtatcagcagaaaccagggaaagcccctaagctcctgatctattatgatgccgaccggccctcaggggtcccatcaaggttcagtggcagtaattctgggaatgatgccactctcaccatcagcagtctgcaacctgaagattttgcaacttactactgtcaagcgccaaccaccaacgagccttataccttcggccagggcaccaaggtggaaatcaagcggacc

SEQ ID NO: 38 - protein, 110 aa, synthetic construct
  REGION 1..110: note = VL
DIQMTQSPSSLSASVGDRVTITCRADNLGDVNVHWYQQKPGKAPKLLIYYDADRPSGVPSRFSGSNSGNDATLTISSLQPEDFATYYCQAPTTNEPYTFGQGTKVEIKRT

SEQ ID NO: 39 - DNA, 363 bp, synthetic construct; identical to SEQ ID NO: 31
  misc_feature 1..363: note = VH
  source 1..363: mol_type = other DNA

SEQ ID NO: 40 - protein, 121 aa, synthetic construct; identical to SEQ ID NO: 32
  REGION 1..121: note = VH

SEQ ID NO: 41 - DNA, 330 bp, synthetic construct
  misc_feature 1..330: note = VL
  source 1..330: mol_type = other DNA
gacatccagatgacccagtctccatcctccctgtctgcatctgtaggagacagagtcaccatcacttgccgggcagataaccttggagatgtaaatgtacactggtatcagcagaaaccagggaaagcccctaagctcctgatctattatgatgccgaccggccctcaggggtcccatcaaggttcagtggcagtaattctgggaatgatgccactctcaccatcagcagtctgcaacctgaagattttgcaacttactactgtcaagcaccaacaaacaacgatccttataccttcggccagggcaccaaggtggaaatcaagcggacc

SEQ ID NO: 42 - protein, 110 aa, synthetic construct
  REGION 1..110: note = VL
DIQMTQSPSSLSASVGDRVTITCRADNLGDVNVHWYQQKPGKAPKLLIYYDADRPSGVPSRFSGSNSGNDATLTISSLQPEDFATYYCQAPTNNDPYTFGQGTKVEIKRT

SEQ ID NO: 43 - DNA, 363 bp, synthetic construct; identical to SEQ ID NO: 31
  misc_feature 1..363: note = VH
  source 1..363: mol_type = other DNA

SEQ ID NO: 44 - protein, 121 aa, synthetic construct; identical to SEQ ID NO: 32
  REGION 1..121: note = VH

SEQ ID NO: 45 - DNA, 330 bp, synthetic construct
  misc_feature 1..330: note = VL
  source 1..330: mol_type = other DNA
gacatccagatgacccagtctccatcctccctgtctgcatctgtaggagacagagtcaccatcacttgccgggcagataaccttggagatgtaaatgtacactggtatcagcagaaaccagggaaagcccctaagctcctgatctattatgatgccgaccggccctcaggggtcccatcaaggttcagtggcagtaattctgggaatgatgccactctcaccatcagcagtctgcaacctgaagattttgcaacttactactgtcaagcaccaaccacgcatctgccttataccttcggccagggtaccaaggtggaaatcaagcggacc

SEQ ID NO: 46 - protein, 110 aa, synthetic construct
  REGION 1..110: note = VL
DIQMTQSPSSLSASVGDRVTITCRADNLGDVNVHWYQQKPGKAPKLLIYYDADRPSGVPSRFSGSNSGNDATLTISSLQPEDFATYYCQAPTTHLPYTFGQGTKVEIKRT

SEQ ID NO: 47 - DNA, 363 bp, synthetic construct; identical to SEQ ID NO: 31
  misc_feature 1..363: note = VH
  source 1..363: mol_type = other DNA

SEQ ID NO: 48 - protein, 121 aa, synthetic construct; identical to SEQ ID NO: 32
  REGION 1..121: note = VH

SEQ ID NO: 49 - DNA, 330 bp, synthetic construct
  misc_feature 1..330: note = VL
  source 1..330: mol_type = other DNA
gacatccagatgacccagtctccatcctccctgtctgcatctgtaggagacagagtcaccatcacttgccgggcagataaccttggagatgtaaatgtacactggtatcagcagaaaccagggaaagcccctaagctcctgatctattatgatgccgaccggccctcaggggtcccatcaaggttcagtggcagtaattctgggaatgatgccactctcaccatcagcagtctgcaacctgaagattttgcaacttactactgtcaagcgccaaccaaaaacgtcccttataccttcggccagggcaccaaggtggaaatcaagcggacc

SEQ ID NO: 50 - protein, 110 aa, synthetic construct
  REGION 1..110: note = VL
DIQMTQSPSSLSASVGDRVTITCRADNLGDVNVHWYQQKPGKAPKLLIYYDADRPSGVPSRFSGSNSGNDATLTISSLQPEDFATYYCQAPTKNVPYTFGQGTKVEIKRT